European Patent Specification EP 3 960 184 B1, published September 11, 2024. Title: Preeclampsia. Applicant: Aston University. The sequence listing filed with the application follows.

SEQUENCE LISTING (29 sequences)

SEQ ID NO: 1 - RNA, 22 nt, Homo sapiens
uggagugugacaaugguguuug

SEQ ID NO: 2 - RNA, 22 nt, Homo sapiens
auauaauacaaccugcuaagug

SEQ ID NO: 3 - RNA, 21 nt, Homo sapiens
ucagugcaugacagaacuugg

SEQ ID NO: 4 - RNA, 21 nt, Homo sapiens
uagcagcacagaaauauuggc

SEQ ID NO: 5 - RNA, 22 nt, Homo sapiens
caaacaccauugucacacucca

SEQ ID NO: 6 - RNA, 22 nt, Homo sapiens
cacuuagcagguuguauuauau

SEQ ID NO: 7 - RNA, 21 nt, Homo sapiens
ccaaguucugucaugcacuga

SEQ ID NO: 8 - RNA, 21 nt, Homo sapiens
gccaauauuucugugcugcua

SEQ ID NO: 9 - DNA, 23 bp, Homo sapiens
tttgtagcattgtcatcactcct

SEQ ID NO: 10 - DNA, 20 bp, Homo sapiens
tttgtcgacggatagagaat

SEQ ID NO: 11 - DNA, 20 bp, Homo sapiens
gtcaaaatagattattataa

SEQ ID NO: 12 - DNA, 17 bp, Homo sapiens
gtcaagagcaaggcgca

SEQ ID NO: 13 - DNA, 22 bp, Homo sapiens
tacaatatttgtactattatat

SEQ ID NO: 14 - DNA, 19 bp, Homo sapiens
tacaatatttagacgcgct

SEQ ID NO: 15 - DNA, 21 bp, Homo sapiens
tccctcccccccatgctgtgg

SEQ ID NO: 16 - DNA, 21 bp, Homo sapiens
tgtaaacaagggtccacagca

SEQ ID NO: 17 - DNA, 45 bp, Homo sapiens
ctctcaggagtagagtacctgtaaaggagaatctctaaatcaagt

SEQ ID NO: 18 - DNA, 45 bp, Homo sapiens
acttgatttagagattctcctttacaggtactctactcctgagag

SEQ ID NO: 19 - RNA, 22 nt, Homo sapiens
guuugugguaacagugugaggu

SEQ ID NO: 20 - RNA, 23 nt, Homo sapiens
uuuguagcauugucaucacuccu

SEQ ID NO: 21 - RNA, 22 nt, Homo sapiens
gugaaucguccaacauaauaua

SEQ ID NO: 22 - RNA, 20 nt, Homo sapiens
gucaaaauagauuauuauaa

SEQ ID NO: 23 - RNA, 21 nt, Homo sapiens
gguucaagacaguacgugacu

SEQ ID NO: 24 - RNA, 21 nt, Homo sapiens
ucccucccccccaugcacugu

SEQ ID NO: 25 - DNA, 16 bp, Mus musculus
taaagtctaatctcta

SEQ ID NO: 26 - DNA, 21 bp, Macaca mulatta
acctgtaaagtctaatctcta

SEQ ID NO: 27 - DNA, 21 bp, Gorilla gorilla
acctgtaaagtctaatctcta

SEQ ID NO: 28 - DNA, 21 bp, Pan troglodytes
acctgtaaagtctaatctcta

SEQ ID NO: 29 - DNA, 21 bp, Homo sapiens
acctgtaaagtctaatctcta